European Patent Specification EP 3 750 995 B1, published December 25, 2024. Title: Peptide Nucleic Acid Complex with Endosome Escape Ability and Uses thereof. Applicant: Seasun Therapeutics, Inc. The sequence listing filed with the application follows.

SEQUENCE LISTING (86 sequences)

SEQ ID NO: 1 - DNA, 15 bp, Artificial Sequence
  PNA
atgattctgccctcc

SEQ ID NO: 2 - DNA, 15 bp, Artificial Sequence
  PNA
atgattctgccctcc

SEQ ID NO: 3 - DNA, 15 bp, Artificial Sequence
  PNA
atgattctgccctcc

SEQ ID NO: 4 - DNA, 5 bp, Artificial Sequence
  PNA
ggagg

SEQ ID NO: 5 - DNA, 5 bp, Artificial Sequence
  PNA
ggagg

SEQ ID NO: 6 - DNA, 5 bp, Artificial Sequence
  PNA
ggagg

SEQ ID NO: 7 - DNA, 15 bp, Artificial Sequence
  PNA
tactaagacgggagg

SEQ ID NO: 8 - DNA, 15 bp, Artificial Sequence
  PNA
tactaagacgggagg

SEQ ID NO: 9 - DNA, 15 bp, Artificial Sequence
  PNA
tactaagacgggagg

SEQ ID NO: 10 - DNA, 14 bp, Artificial Sequence
  PNA
atgaaagcaatgat

SEQ ID NO: 11 - DNA, 5 bp, Artificial Sequence
  PNA
atcat

SEQ ID NO: 12 - DNA, 15 bp, Artificial Sequence
  PNA
tcaatagtgcaatca

SEQ ID NO: 13 - DNA, 15 bp, Artificial Sequence
  PNA
ctcaatggcttccag

SEQ ID NO: 14 - DNA, 15 bp, Artificial Sequence
  PNA
tcaatagtgcaatca

SEQ ID NO: 15 - DNA, 15 bp, Artificial Sequence
  PNA
ctcaatggcttccag

SEQ ID NO: 16 - DNA, 5 bp, Artificial Sequence
  PNA
tgatt

SEQ ID NO: 17 - DNA, 5 bp, Artificial Sequence
  PNA
ttagt

SEQ ID NO: 18 - DNA, 15 bp, Artificial Sequence
  PNA
tgattgcactattga

SEQ ID NO: 19 - DNA, 15 bp, Artificial Sequence
  PNA
agttatcacgttagt

SEQ ID NO: 20 - DNA, 5 bp, Artificial Sequence
  PNA
tgatt

SEQ ID NO: 21 - DNA, 5 bp, Artificial Sequence
  PNA
ttagt

SEQ ID NO: 22 - DNA, 15 bp, Artificial Sequence
  PNA
tgattgcactattga

SEQ ID NO: 23 - DNA, 15 bp, Artificial Sequence
  PNA
agttatcacgttagt

SEQ ID NO: 24 - DNA, 5 bp, Artificial Sequence
  PNA
ctgga

SEQ ID NO: 25 - DNA, 5 bp, Artificial Sequence
  PNA
aggtc

SEQ ID NO: 26 - DNA, 15 bp, Artificial Sequence
  PNA
ctggaagccattgag

SEQ ID NO: 27 - DNA, 15 bp, Artificial Sequence
  PNA
gagttaccgaaggtc

SEQ ID NO: 28 - DNA, 6 bp, Artificial Sequence
  PNA
kctgga

SEQ ID NO: 29 - DNA, 5 bp, Artificial Sequence
  PNA
aggtc

SEQ ID NO: 30 - DNA, 15 bp, Artificial Sequence
  PNA
ctggaagccattgag

SEQ ID NO: 31 - DNA, 14 bp, Artificial Sequence
  PNA
gagttaccgaagtc

SEQ ID NO: 32 - DNA, 17 bp, Artificial Sequence
  PNA
tactcaagctacattca

SEQ ID NO: 33 - DNA, 14 bp, Artificial Sequence
  PNA
gagccacttctgca

SEQ ID NO: 34 - DNA, 17 bp, Artificial Sequence
  PNA
tactcaagctacattca

SEQ ID NO: 35 - DNA, 14 bp, Artificial Sequence
  PNA
gagccacttctgca

SEQ ID NO: 36 - DNA, 5 bp, Artificial Sequence
  PNA
atgtc

SEQ ID NO: 37 - DNA, 5 bp, Artificial Sequence
  PNA
ctgta

SEQ ID NO: 38 - DNA, 15 bp, Artificial Sequence
  PNA
atgtccaatcaggga

SEQ ID NO: 39 - DNA, 15 bp, Artificial Sequence
  PNA
agggactaacctgta

SEQ ID NO: 40 - DNA, 5 bp, Artificial Sequence
  PNA
atgtc

SEQ ID NO: 41 - DNA, 5 bp, Artificial Sequence
  PNA
ctgta

SEQ ID NO: 42 - DNA, 15 bp, Artificial Sequence
  PNA
atgtccaatcaggga

SEQ ID NO: 43 - DNA, 15 bp, Artificial Sequence
  PNA
agggactaacctgta

SEQ ID NO: 44 - DNA, 5 bp, Artificial Sequence
  PNA
tgcag

SEQ ID NO: 45 - DNA, 5 bp, Artificial Sequence
  PNA
gacgt

SEQ ID NO: 46 - DNA, 14 bp, Artificial Sequence
  PNA
tgcagaagtggctc

SEQ ID NO: 47 - DNA, 14 bp, Artificial Sequence
  PNA
ctcggtgaagacgt

SEQ ID NO: 48 - DNA, 5 bp, Artificial Sequence
  PNA
tgcag

SEQ ID NO: 49 - DNA, 5 bp, Artificial Sequence
  PNA
gacgt

SEQ ID NO: 50 - DNA, 14 bp, Artificial Sequence
  PNA
tgcagaagtggctc

SEQ ID NO: 51 - DNA, 14 bp, Artificial Sequence
  PNA
ctcggtgaagacgt

SEQ ID NO: 52 - DNA, 17 bp, Artificial Sequence
  PNA
tactcaagctacattca

SEQ ID NO: 53 - DNA, 16 bp, Artificial Sequence
  PNA
tccacatcaaagcact

SEQ ID NO: 54 - DNA, 17 bp, Artificial Sequence
  PNA
tactcaagctacattca

SEQ ID NO: 55 - DNA, 16 bp, Artificial Sequence
  PNA
tccacatcaaagcact

SEQ ID NO: 56 - DNA, 5 bp, Artificial Sequence
  PNA
tcaat

SEQ ID NO: 57 - DNA, 17 bp, Artificial Sequence
  PNA
atgagttcgatgtaagt

SEQ ID NO: 58 - DNA, 5 bp, Artificial Sequence
  PNA
tcaat

SEQ ID NO: 59 - DNA, 17 bp, Artificial Sequence
  PNA
atgagttcgatgtaagt

SEQ ID NO: 60 - DNA, 5 bp, Artificial Sequence
  PNA
agtgc

SEQ ID NO: 61 - DNA, 16 bp, Artificial Sequence
  PNA
aggtgtagtttcgtga

SEQ ID NO: 62 - DNA, 5 bp, Artificial Sequence
  PNA
agtgc

SEQ ID NO: 63 - DNA, 16 bp, Artificial Sequence
  PNA
aggtgtagtttcgtga

SEQ ID NO: 64 - DNA, 17 bp, Artificial Sequence
  PNA
atgtaggtgatcctgtt

SEQ ID NO: 65 - DNA, 17 bp, Artificial Sequence
  PNA
atgtaggtgatcctgtt

SEQ ID NO: 66 - DNA, 5 bp, Artificial Sequence
  PNA
aacag

SEQ ID NO: 67 - DNA, 5 bp, Artificial Sequence
  PNA
aacag

SEQ ID NO: 68 - DNA, 5 bp, Artificial Sequence
  PNA
gacaa

SEQ ID NO: 69 - DNA, 17 bp, Artificial Sequence
  PNA
tacatccactaggacaa

SEQ ID NO: 70 - DNA, 17 bp, Artificial Sequence
  PNA
tacaggatcacctacat

SEQ ID NO: 71 - DNA, 17 bp, Artificial Sequence
  PNA
tacatccactaggacaa

SEQ ID NO: 72 - DNA, 15 bp, Artificial Sequence
  PNA
tgtcaagccactgca

SEQ ID NO: 73 - DNA, 15 bp, Artificial Sequence
  PNA
tgtcaagccactgca

SEQ ID NO: 74 - DNA, 5 bp, Artificial Sequence
  PNA
tgcag

SEQ ID NO: 75 - DNA, 5 bp, Artificial Sequence
  PNA
tgcag

SEQ ID NO: 76 - DNA, 15 bp, Artificial Sequence
  PNA
acagttcggtgacgt

SEQ ID NO: 77 - DNA, 15 bp, Artificial Sequence
  PNA
tgcagtggcttgaca

SEQ ID NO: 78 - DNA, 15 bp, Artificial Sequence
  PNA
acagttcggtgacgt

SEQ ID NO: 79 - DNA, 15 bp, Artificial Sequence
  PNA
gcttctacagcttca

SEQ ID NO: 80 - DNA, 15 bp, Artificial Sequence
  PNA
gcttctacagcttca

SEQ ID NO: 81 - DNA, 5 bp, Artificial Sequence
  PNA
tgaag

SEQ ID NO: 82 - DNA, 5 bp, Artificial Sequence
  PNA
tgaag

SEQ ID NO: 83 - DNA, 15 bp, Artificial Sequence
  PNA
tgaagctgtagaagc

SEQ ID NO: 84 - DNA, 15 bp, Artificial Sequence
  PNA
tgaagctgtagaagc

SEQ ID NO: 85 - protein, 26 aa, Artificial Sequence
  peptide
GIGAVLKVLTTGLPALISWIKRKRQQ

SEQ ID NO: 86 - protein, 13 aa, Artificial Sequence
  peptide
GLFDIIKKIAESF